European Patent Application EP 4 212 551 A1, published July 19, 2023. Title: Antibody Binding to human IL-5R alpha and Uses Thereof. Applicant: Ajou University Industry-Academic Cooperation Foundation. The sequence listing filed with the application follows.

SEQUENCE LISTING (32 sequences)

SEQ ID NO: 1 - protein, 122 aa, Artificial Sequence
  m2B7 VH
QVQLQQPGAELVRPGASVKLSCKASGYTFTSYWINWVKQRPGQGLEWIGHIYPSESYTNYNQKFKDKATLTVDKSSSTAYMQLSSPTSEDSAVYYCTRDYYGRSYYYAMDYWGQGTSVTVSS

SEQ ID NO: 2 - protein, 122 aa, Artificial Sequence
  hu2B7 VH
QVQLVQSGAEVKKPGSSVKVSCKASGYTFTSYWINWVRQAPGQGLEWIGHIYPSESYTNYNQKFKDKATLTVDKSTNTAYMELSSLRSEDTAVYYCTRDYYGRSYYYAMDYWGQGTTLTVSS

SEQ ID NO: 3 - protein, 5 aa, Artificial Sequence
  Synthetic CDR1 Sequence
SYWIN

SEQ ID NO: 4 - protein, 17 aa, Artificial Sequence
  Synthetic CDR2 Sequence
HIYPSESYTNYNQKFKD

SEQ ID NO: 5 - protein, 13 aa, Artificial Sequence
  Synthetic CDR3 Sequence
DYYGRSYYYAMDY

SEQ ID NO: 6 - protein, 107 aa, Artificial Sequence
  m2B7 VL
DIVMTQSHKFMSTSVGDRVSITCKASQNVGTAVAWYQQKPGQSPKLLIYWASTRHTGVPDRFTGSGSGTDFTFTISNVQSEDLADYFCQQFGRYPYTFGGGTKLEIK

SEQ ID NO: 7 - protein, 107 aa, Artificial Sequence
  hu2B7 VL
DIQMTQSPSTLSASVGDRVTITCKASQNVGTAVAWYQQKPGKAPKLLIYWASTRHTGVPDRFSGSGSGTDFTLTISSLQPDDFATYYCQQFGRYPYTFGSGTKVEVK

SEQ ID NO: 8 - protein, 27 aa, Artificial Sequence
  Synthetic CDR1 Sequence
KASQNVGTAVAWASTRHTQQFGRYPYT

SEQ ID NO: 9 - protein, 7 aa, Artificial Sequence
  Synthetic CDR2 Sequence
WASTRHT

SEQ ID NO: 10 - protein, 9 aa, Artificial Sequence
  Synthetic CDR3 Sequence
QQFGRYPYT

SEQ ID NO: 11 - protein, 122 aa, Artificial Sequence
  VH
QVQLVQSGAEVKKPGSSVKVSCKASGYTFTSYWINWVRQAPGQGLEWIGHIYPNKNENYYNHKFKDKATLTVDKSTNTAYMELSSLRSEDTAVYYCTRDYYGRSYYYAMDYWGQGTTLTVSS

SEQ ID NO: 12 - protein, 122 aa, Artificial Sequence
  VH
QVQLVQSGAEVKKPGSSVKVSCKASGYTFTSYWINWVRQAPGQGLEWIGHIYPTATIAVYNDKFKDKATLTVDKSTNTAYMELSSLRSEDTAVYYCTRDYYGRSYYYAMDYWGQGTTLTVSS

SEQ ID NO: 13 - protein, 122 aa, Artificial Sequence
  VH
QVQLVQSGAEVKKPGSSVKVSCKASGYTFTSYWINWVRQAPGQGLEWIGHIYPQKTLTIYNHKFKDKATLTVDKSTNTAYMELSSLRSEDTAVYYCTRDYYGRSYYYAMDYWGQGTTLTVSS

SEQ ID NO: 14 - protein, 122 aa, Artificial Sequence
  VH
QVQLVQSGAEVKKPGSSVKVSCKASGYTFTSYWINWVRQAPGQGLEWIGHIYPTSSVKFYNNKFKDKATLTVDKSTNTAYMELSSLRSEDTAVYYCTRDYYGRSYYYAMDYWGQGTTLTVSS

SEQ ID NO: 15 - protein, 17 aa, Artificial Sequence
  Synthetic CDR2 Sequence
HIYPNKNENYYNHKFKD

SEQ ID NO: 16 - protein, 17 aa, Artificial Sequence
  Synthetic CDR2 Sequence
HIYPTATIAVYNDKFKD

SEQ ID NO: 17 - protein, 17 aa, Artificial Sequence
  Synthetic CDR2 Sequence
HIYPQKTLTIYNHKFKD

SEQ ID NO: 18 - protein, 17 aa, Artificial Sequence
  Synthetic CDR2 Sequence
HIYPTSSVKFYNNKFKD

SEQ ID NO: 19 - protein, 322 aa, Artificial Sequence
  IL-5R alpha
DLLPDEKISLLPPVNFTIKVTGLAQVLLQWKPNPDQEQRNVNLEYQVKINAPKEDDYETRITESKCVTILHKGFSASVRTILQNDHSLLASSWASAELHAPPGSPGTSIVNLTCTTNTTEDNYSRLRSYQVSLHCTWLVGTDAPEDTQYFLYYRYGSWTEECQEYSKDTLGRNIACWFPRTFILSKGRDWLAVLVNGSSKHSAIRPFDQLFALHAIDQINPPLNVTAEIEGTRLSIQWEKPVSAFPIHCFDYEVKIHNTRNGYLQIEKLMTNAFISIIDDLSKYDVQVRAAVSSMCREAGLWSEWSQPIYVGNDEHKPLREW

SEQ ID NO: 20 - protein, 321 aa, Artificial Sequence
  mIL-5R alpha D1
DLLNHKKFLLLPPVNFTIKATGLAQVLLHWDPNPDQEQRHVDLEYHVKINAPQEDEYDTRKTESKCVTPLHEGFAASVRTILKSSHTTLASSWVSAELKAPPGSPGTSVTNLTCTTHTVVSSHTHLRPYQVSLRCTWLVGKDAPEDTQYFLYYRFGVLTEKCQEYSRDALNRNTACWFPRTFINSKGFEQLAVHINGSSKRAAIKPFDQLFSPLAIDQVNPPRNVTVEIESNSLYIQWEKPLSAFPDHCFNYELKIYNTKNGHIQKEKLIANKFISKIDDVSTYSIQVRAAVSSPCRMPGRWGEWSQPIYVGKERKSLVEW

SEQ ID NO: 21 - protein, 122 aa, Artificial Sequence
  VH
QVQLVQSGAEVKKPGSSVKVSCKASGYTFTSYWINWVRQAPGQGLEWIGHIYPNKNENYYNHKFKDKATLTVDKSTNTAYMELSSLRSEDTAVYYCTREFYGRQYYQAMDYWGQGTTLTVSS

SEQ ID NO: 22 - protein, 122 aa, Artificial Sequence
  VH
QVQLVQSGAEVKKPGSSVKVSCKASGYTFTSYWINWVRQAPGQGLEWIGHIYPNKNENYYNHKFKDKATLTVDKSTNTAYMELSSLRSEDTAVYYCTREYYGRSYYAAMDYWGQGTTLTVSS

SEQ ID NO: 23 - protein, 122 aa, Artificial Sequence
  VH
QVQLVQSGAEVKKPGSSVKVSCKASGYTFTSYWINWVRQAPGQGLEWIGHIYPNKNENYYNHKFKDKATLTVDKSTNTAYMELSSLRSEDTAVYYCTREHYGRPYYNAMDYWGQGTTLTVSS

SEQ ID NO: 24 - protein, 122 aa, Artificial Sequence
  VH
QVQLVQSGAEVKKPGSSVKVSCKASGYTFTSYWINWVRQAPGQGLEWIGHIYPNKNENYYNHKFKDKATLTVDKSTNTAYMELSSLRSEDTAVYYCTREYYGRTYYSAMDYWGQGTTLTVSS

SEQ ID NO: 25 - protein, 122 aa, Artificial Sequence
  VH
QVQLVQSGAEVKKPGSSVKVSCKASGYTFTSYWINWVRQAPGQGLEWIGHIYPNKNENYYNHKFKDKATLTVDKSTNTAYMELSSLRSEDTAVYYCTREFYGRSRYSAMDYWGQGTTLTVSS

SEQ ID NO: 26 - protein, 122 aa, Artificial Sequence
  VH
QVQLVQSGAEVKKPGSSVKVSCKASGYTFTSYWINWVRQAPGQGLEWIGHIYPNKNENYYNHKFKDKATLTVDKSTNTAYMELSSLRSEDTAVYYCTREYYGRSYYNAMDYWGQGTTLTVSS

SEQ ID NO: 27 - protein, 13 aa, Artificial Sequence
  CDR3
EFYGRQYYQAMDY

SEQ ID NO: 28 - protein, 13 aa, Artificial Sequence
  CDR3
EYYGRSYYAAMDY

SEQ ID NO: 29 - protein, 13 aa, Artificial Sequence
  CDR3
EHYGRPYYNAMDY

SEQ ID NO: 30 - protein, 13 aa, Artificial Sequence
  CDR3
EYYGRTYYSAMDY

SEQ ID NO: 31 - protein, 13 aa, Artificial Sequence
  CDR3
EFYGRSRYSAMDY

SEQ ID NO: 32 - protein, 13 aa, Artificial Sequence
  CDR3
EYYGRSYYNAMDY